European Patent Application EP 4 461 313 A1, published November 13, 2024. Title: Pharmaceutical composition for treatmenting cancer. Applicant: Fujiwara, Hiroshi. The sequence listing filed with the application follows.

SEQUENCE LISTING (31 sequences)

SEQ ID NO: 1 - protein, 8 aa, mouse
GYSFTDYI

SEQ ID NO: 2 - protein, 8 aa, mouse
INPYHAGI

SEQ ID NO: 3 - protein, 13 aa, mouse
ARGSNYVYYYAMD

SEQ ID NO: 4 - protein, 5 aa, mouse
SSVSY

SEQ ID NO: 5 - protein, 9 aa, mouse
QQWSSNPPT

SEQ ID NO: 6 - protein, 477 aa, mouse
MSSPQPLKTLTLTMGGSWIFLFLLSGTAGAHSEIQLQQTGPELVKPGASVKISCKASGYSFTDYIMLWVKQSHGKSLEWIGNINPYHAGISYNLKFKGKATLTVDTSSSTAYMQLNSLTSEDSAVYYCARGSNYVYYYAMDYWGQGTSVTVSSAKTTPPSVYPLAPGSAAQTNSMVTLGCLVKGYFPEPVTVTWNSGSLSSGVHTFPAVLQSDLYTLSSSVTVPSSTWPSETVTCNVAHPASSTKVDKKIVPRDCGCKPCICTVPEVSSVFIFPPKPKDVLTITLTPKVTCVVVDISKDDPEVQFSWFVDDVEVHTAQTQPREEQFNSTFRSVSELPIMHQDWLNGKEFKCRVNSAAFPAPIEKTISKTKGRPKAPQVYTIPPPKEQMAKDKVSLTCMITDFFPEDITVEWQWNGQPAENYKNTQPIMDTDGSYFVYSKLNVQKSNWEAGNTFTCSVLHEGLHNHHTEKSLSHSPGK

SEQ ID NO: 7 - protein, 235 aa, mouse
MDFQVQIFSFLLISASVIMSRGQIVLSQSPAILSASPGEKVTMTCRASSSVSYMHWYQQKPGSSPKPWIFATSNLASGVPARFSGSGSGTSYSLTISRVEAEDAATYYCQQWSSNPPTFGGGTKLEIKRADAAPTVSIFPPSSEQLTSGGASVVCFLNNFYPKDINVKWKIDGSERQNGVLNSWTDQDSKDSTYSMSSTLTLTKDEYERHNSYTCEATHKTSTSPIVKSFNRNEC

SEQ ID NO: 8 - DNA, 1431 bp, mouse
  source 1..1431: mol_type = other DNA
atgtcctctccacagcccctgaagacactgactctaaccatgggagggagctggatctttctcttcctcctgtcaggaactgcaggtgcccactctgagatccagctgcagcagactggacctgagctggtgaagcctggggcttcagtgaagatatcctgcaaggcttccggttattcattcactgactacatcatgctctgggtgaagcagagccatggaaagagccttgagtggattggaaatattaatccttaccatgctggtattagctacaatctgaagttcaagggcaaggccacattgactgtagacacatcttccagcacagcctacatgcagctcaacagtctgacatctgaggactctgcagtctattactgtgcaagagggagtaattacgtctattactatgctatggactactggggtcaaggaacctcagtcaccgtctcctcagccaaaacgacacccccatctgtctatccactggcccctggatctgctgcccaaactaactccatggtgaccctgggatgcctggtcaagggctatttccctgagccagtgacagtgacctggaactctggatccctgtccagcggtgtgcacaccttcccagctgtcctgcagtctgacctctacactctgagcagctcagtgactgtcccctccagcacctggcccagcgagaccgtcacctgcaacgttgcccacccggccagcagcaccaaggtggacaagaaaattgtgcccagggattgtggttgtaagccttgcatatgtacagtcccagaagtatcatctgtcttcatcttccccccaaagcccaaggatgtgctcaccattactctgactcccaaggtcacgtgtgttgtggtagacatcagcaaggatgatcccgaggtccagttcagctggtttgtagatgatgtggaggtgcacacagctcagacgcaaccccgggaggagcagttcaacagcactttccgctcagtcagtgaacttcccatcatgcaccaggactggctcaatggcaaggagttcaaatgcagggtcaacagtgcagctttccctgcccccatcgagaaaaccatctccaaaaccaaaggcagaccgaaggctccacaggtgtacaccattccacctcccaaggagcagatggccaaggataaagtcagtctgacctgcatgataacagacttcttccctgaagacattactgtggagtggcagtggaatgggcagccagcggagaactacaagaacactcagcccatcatggacacagatggctcttacttcgtctacagcaagctcaatgtgcagaagagcaactgggaggcaggaaatactttcacctgctctgtgttacatgagggcctgcacaaccaccatactgagaagagcctctcccactctcctggtaaa

SEQ ID NO: 9 - DNA, 705 bp, mouse
  source 1..705: mol_type = other DNA
atggattttcaagtgcagattttcagcttcctgctaatcagtgcttcagtcataatgtccagaggacaaattgttctctcccagtctccagcaattctgtctgcatctccaggggagaaggtcacaatgacttgcagggccagttcaagtgtaagttacatgcactggtatcagcagaagccaggatcctcccccaaaccctggatttttgccacatccaacctggcttctggagtccctgctcgcttcagtggcagtgggtctgggacctcttattctctcacaatcagcagagtggaggctgaagatgctgccacttattactgccagcagtggagtagtaacccaccgacgttcggtggaggcaccaagctggaaatcaaacgggctgatgctgcaccaactgtatccatcttcccaccatccagtgagcagttaacatctggaggtgcctcagtcgtgtgcttcttgaacaacttctaccccaaagacatcaatgtcaagtggaagattgatggcagtgaacgacaaaatggcgtcctgaacagttggactgatcaggacagcaaagacagcacctacagcatgagcagcaccctcacgttgaccaaggacgagtatgaacgacataacagctatacctgtgaggccactcacaagacatcaacttcacccattgtcaagagcttcaacaggaatgagtgt

SEQ ID NO: 10 - protein, 990 aa, homo sapiens [sequence omitted]

SEQ ID NO: 11 - protein, 8 aa, mouse
GYTFTSYW

SEQ ID NO: 12 - protein, 8 aa, mouse
IDPYDSET

SEQ ID NO: 13 - protein, 12 aa, mouse
ARDYGSRYYAMD

SEQ ID NO: 14 - protein, 6 aa, mouse
ENVVTY

SEQ ID NO: 15 - protein, 7 aa, mouse
GQGYSYP

SEQ ID NO: 16 - protein, 5 aa, mouse
STISY

SEQ ID NO: 17 - protein, 8 aa, mouse
QQWSSNPP

SEQ ID NO: 18 - protein, 8 aa, mouse
GYTFTDYY

SEQ ID NO: 19 - protein, 8 aa, mouse
IYPRSGHS

SEQ ID NO: 20 - protein, 12 aa, mouse
QSLLYSNIQKNY

SEQ ID NO: 21 - protein, 7 aa, mouse
QQYYSYP

SEQ ID NO: 22 - protein, 463 aa, mouse
MGWSYIILFLLATATCVHSQVQLQQPGAELVRPGASVKLSCKASGYTFTSYWMNWVRQRPEQGLEWIGRIDPYDSETHYNQKFKDKAILTVDKSSSTVHMQLSSLTSEDSAVYHCARDYGSRYYAMDYWGQGTSVTVSSAKTTPPSVYPLAPGSAAQTNSMVTLGCLVKGYFPEPVTVTWNSGSLSSGVHTFPAVLQSDLYTLSSSVTVPSSTWPSETVTCNVAHPASSTKVDKKIEPRDCGCKPCICTVPEVSSVFIFPPKPKDVLTITLTPKVTCVVVDISKDDPEVQFSWFVDDVEVHTAQTQPREEQFNSTFRSVSELPIMHQDWLNGKEFKCRVNSAAFPAPIEKTISKTKGRPKAPQVYTIPPPKEQMAKDKVSLTCMITDFFPEDITVEWQWNGQPAENYKNTQPIMDTDGSYFVYSKLNVQKSNWEAGNTFTCSVLHEGLHNHHTEKSLSHSPGK

SEQ ID NO: 23 - protein, 238 aa, mouse
MGIKMESQTLVFISILLWLYGADGNIVMTQSPKSMSMSVGERVTLTCKASENVVTYVSWYQQKPEQSPKLLIYGASNRYTGVPDRFTGSGSATDFTLTISSVQAEDLADYHCGQGYSYPYTFGGGTKLEIKRADAAPTVSIFPPSSEQLTSGGASVVCFLNNFYPKDINVKWKIDGSERQNGVLNSWTDQDSKDSTYSMSSTLTLTKDEYERHNSYTCEATHKTSTSPIVKSFNRNEC

SEQ ID NO: 24 - protein, 235 aa, mouse
MDFQVQIFSFLLISASVIISRGQIVLTQSPTIMSVSPGEKVTMTCSASSTISYMHWYQQKSGTSPKRWIYDTSKLASGVPARFSGSGSGTSYSLTITSMGAEDAATYYCQQWSSNPPTFGGGTKLEIKRADAAPTVSIFPPSSEQLTSGGASVVCFLNNFYPKDINVKWKIDGSERQNGVLNSWTDQDSKDSTYSMSSTLTLTKDEYERHNSYTCEATHKTSTSPIVKSFNRNEC

SEQ ID NO: 25 - protein, 475 aa, mouse
MEWIWIFLFILSGTAGVHSQVQLQQSGAELAGPGTSVRLSCKASGYTFTDYYIDWVKQRTGQGLEWIGEIYPRSGHSKYNEKFEGKATLTADKSSSTAYMHLSSLTSEDSAVYFCALYYYGSSHWFAYWGQGTLVTVSAAKTTPPSVYPLAPGSAAQTNSMVTLGCLVKGYFPEPVTVTWNSGSLSSGVHTFPAVLQSDLYTLSSSVTVPSSTWPSETVTCNVAHPASSTTVDKKLEPSGPISTINPCPPCKECHKCPAPNLEGGPSVFIFPPNIKDVLMISLTPKVTCVVVDVSEDDPDVQISWFVNNVEVHTAQTQTHREDYNSTIRVVSTLPIQHQDWMSGKEFKCKVNNKDLPSPIERTISKIKGLVRAPQVYILPPPAEQLSRKDVSLTCLVVGFNPGDISVEWTSNGHTEENYKDTAPVLDSDGSYFIYSKLNMKTSKWEKTDSFSCNVRHEGLKNYYLKKTISRSPGK

SEQ ID NO: 26 - protein, 240 aa, mouse
MDSQAQVLMLLLLWVSGTCGDIVMSQSPSSLTVSVGERVTMSCRSSQSLLYSNIQKNYLAWYQQKPGQSPKLLIYWASTRESGVPDRFTGSGSGTDFTLTISSVKAEDLAVYYCQQYYSYPYTFGGGTKLEIKRADAAPTVSIFPPSSEQLTSGGASVVCFLNNFYPKDINVKWKIDGSERQNGVLNSWTDQDSKDSTYSMSSTLTLTKDEYERHNSYTCEATHKTSTSPIVKSFNRNEC

SEQ ID NO: 27 - DNA, 1389 bp, mouse
  source 1..1389: mol_type = other DNA
atgggatggagctatatcatcctcttcttgttagcaacagctacatgtgtccactcccaggtccaactgcagcagcctggggctgagctggtgaggcctggggcttcagtgaagctgtcctgcaaggcttctggctacacgttcaccagctactggatgaactgggttaggcagaggcctgagcaaggccttgagtggattggaaggattgatccttacgatagtgaaactcactacaatcaaaagttcaaggacaaggccattttgactgtagacaaatcctccagtacagtccacatgcaactaagcagcctgacatctgaggactctgcggtctatcactgtgcaagagactacggtagtaggtactatgctatggactactggggtcaaggaacctcagtcaccgtctcctcagccaaaacgacacccccatctgtctatccactggcccctggatctgctgcccaaactaactccatggtgaccctgggatgcctggtcaagggctatttccctgagccagtgacagtgacctggaactctggatccctgtccagcggtgtgcacaccttcccagctgtcctgcagtctgacctctacactctgagcagctcagtgactgtcccctccagcacctggcccagcgagaccgtcacctgcaacgttgcccacccggccagcagcaccaaggtggacaagaaaattgtgcccagggattgtggttgtaagccttgcatatgtacagtcccagaagtatcatctgtcttcatcttccccccaaagcccaaggatgtgctcaccattactctgactcccaaggtcacgtgtgttgtggtagacatcagcaaggatgatcccgaggtccagttcagctggtttgtagatgatgtggaggtgcacacagctcagacgcaaccccgggaggagcagttcaacagcactttccgctcagtcagtgaacttcccatcatgcaccaggactggctcaatggcaaggagttcaaatgcagggtcaacagtgcagctttccctgcccccatcgagaaaaccatctccaaaaccaaaggcagaccgaaggctccacaggtgtacaccattccacctcccaaggagcagatggccaaggataaagtcagtctgacctgcatgataacagacttcttccctgaagacattactgtggagtggcagtggaatgggcagccagcggagaactacaagaacactcagcccatcatggacacagatggctcttacttcgtctacagcaagctcaatgtgcagaagagcaactgggaggcaggaaatactttcacctgctctgtgttacatgagggcctgcacaaccaccatactgagaagagcctctcccactctcctggtaaa

SEQ ID NO: 28 - DNA, 714 bp, mouse
  source 1..714: mol_type = other DNA
atgggcatcaagatggaatcacagactctggtcttcatatccatactgctctggttatatggagctgatgggaacattgtaatgacccaatctcccaaatccatgtccatgtcagtaggagagagggtcaccttgacctgcaaggccagtgagaatgtggttacttatgtttcctggtatcaacagaaaccagagcagtctcctaaactgctgatatacggggcatccaaccggtacactggggtccccgatcgcttcacaggcagtggatctgcaacagatttcactctgaccatcagcagtgtgcaggctgaagaccttgcagattatcactgtggacagggttacagctatccgtacacgttcggaggggggaccaagctggaaataaaacgggctgatgctgcaccaactgtatccatcttcccaccatccagtgagcagttaacatctggaggtgcctcagtcgtgtgcttcttgaacaacttctaccccaaagacatcaatgtcaagtggaagattgatggcagtgaacgacaaaatggcgtcctgaacagttggactgatcaggacagcaaagacagcacctacagcatgagcagcaccctcacgttgaccaaggacgagtatgaacgacataacagctatacctgtgaggccactcacaagacatcaacttcacccattgtcaagagcttcaacaggaatgagtgt

SEQ ID NO: 29 - DNA, 705 bp, mouse
  source 1..705: mol_type = other DNA
atggattttcaagtgcagattttcagcttcctgctaatcagtgcctcagtcataatatccagaggacaaattgttctcacccagtctccaacaatcatgtctgtatctccaggggagaaggtcaccatgacctgcagtgccagctcaactataagttacatgcactggtaccagcagaagtcaggcacctcccccaaaagatggatttatgacacatccaaactggcttctggagtccctgctcgcttcagtggcagtgggtctgggacctcttactctctcacaatcaccagcatgggggctgaagatgctgccacttattactgccagcagtggagtagtaacccacccacgttcggaggggggaccaagctggaaataaaacgggctgatgctgcaccaactgtatccatcttcccaccatccagtgagcagttaacatctggaggtgcctcagtcgtgtgcttcttgaacaacttctaccccaaagacatcaatgtcaagtggaagattgatggcagtgaacgacaaaatggcgtcctgaacagttggactgatcaggacagcaaagacagcacctacagcatgagcagcaccctcacgttgaccaaggacgagtatgaacgacataacagctatacctgtgaggccactcacaagacatcaacttcacccattgtcaagagcttcaacaggaatgagtgt

SEQ ID NO: 30 - DNA, 1425 bp, mouse
  source 1..1425: mol_type = other DNA
atggaatggatctggatctttctcttcatcctctcaggaactgcaggtgtccactcccaggttcagctgcagcagtctggagctgagctggcggggcccgggacttcagtgaggctgtcctgcaaggcttctggctacaccttcactgactactacatagactgggtgaagcagaggactggacagggccttgagtggattggagagatttatcctagaagtggtcattctaagtacaacgagaagttcgagggcaaggccacactgactgcagacaaatcctccagcacagcctacatgcacctcagcagcctgacatctgaagactctgcagtctatttctgtgccctctattactacggcagtagtcactggtttgcttactggggccaagggactctggtcactgtctctgcagccaaaacgacacccccatctgtctatccactggcccctggatctgctgcccaaactaactccatggtgaccctgggatgcctggtcaagggctatttccctgagccagtgacagtgacctggaactctggatccctgtccagcggtgtgcacaccttcccagctgtcctgcagtctgacctctacactctgagcagctcagtgactgtcccctccagcacctggcccagcgagaccgtcacctgcaacgttgcccacccggccagcagcaccacggtggacaaaaaacttgagcccagcgggcccatttcaacaatcaacccctgtcctccatgcaaggagtgtcacaaatgcccagctcctaacctcgagggtggaccatccgtcttcatcttccctccaaatatcaaggatgtactcatgatctccctgacacccaaggtcacgtgtgtggtggtggatgtgagcgaggatgacccagacgtccagatcagctggtttgtgaacaacgtggaagtacacacagctcagacacaaacccatagagaggattacaacagtactatccgggtggtcagcaccctccccatccagcaccaggactggatgagtggcaaggagttcaaatgcaaggtcaacaacaaagacctcccatcacccatcgagagaaccatctcaaaaattaaagggctagtcagagctccacaagtatacatcttgccgccaccagcagagcagttgtccaggaaagatgtcagtctcacttgcctggtcgtgggcttcaaccctggagacatcagtgtggagtggaccagcaacgggcatacagaggagaactacaaggacaccgcaccagtcctggactctgacggttcttacttcatatatagcaagctcaatatgaaaacaagcaagtgggagaaaacagattccttctcatgcaacgtgagacacgagggtctgaaaaattactacctgaagaagaccatctcccggtctccgggtaaa

SEQ ID NO: 31 - DNA, 720 bp, mouse
  source 1..720: mol_type = other DNA
atggattcacaggcccaggttcttatgttactgctgctatgggtatctggtacctgtggggacattgtgatgtcacagtctccatcctccctaactgtgtcagttggagagagggttactatgagctgcaggtccagtcagagccttttatatagtaacattcaaaagaactacttggcctggtaccagcagaaaccggggcagtctcctaaactgctgatttactgggcatccactagggaatctggggtccctgatcgcttcacaggcagtggatctgggacagatttcactctcaccatcagcagtgtgaaggctgaagacctggcagtttattactgtcagcaatattatagctatccgtacacgttcggaggggggaccaagctggaaataaaacgggctgatgctgcaccaactgtatccatcttcccaccatccagtgagcagttaacatctggaggtgcctcagtcgtgtgcttcttgaacaacttctaccccaaagacatcaatgtcaagtggaagattgatggcagtgaacgacaaaatggcgtcctgaacagttggactgatcaggacagcaaagacagcacctacagcatgagcagcaccctcacgttgaccaaggacgagtatgaacgacataacagctatacctgtgaggccactcacaagacatcaacttcacccattgtcaagagcttcaacaggaatgagtgt